European Patent Application EP 4 306 651 A1, published January 17, 2024. Title: COMPOSITION AND THE USE OF CELL LYSIS REAGENTS. Applicant: Vilnius University. Application US. The sequence listing filed with the application follows.

SEQUENCE LISTING (17 sequences)

SEQ ID NO: 1 - DNA, 58 bp, synthetic construct
  source 1..58: mol_type = other DNA
ctacacgacgctcttccgatctnnnnnntttttttttttttttttttttttttttttt

SEQ ID NO: 2 - DNA, 33 bp, synthetic construct
  misc_feature 27..33: note = RNA rgrgrg
  source 1..33: mol_type = other DNA
aagcagtggtatcaacgcagagtacatrgrgrg

SEQ ID NO: 3 - DNA, 23 bp, synthetic construct
  source 1..23: mol_type = other DNA
aagcagtggtatcaacgcagagt

SEQ ID NO: 4 - DNA, 22 bp, synthetic construct
  source 1..22: mol_type = other DNA
ctacacgacgctcttccgatct

SEQ ID NO: 5 - DNA, 19 bp, synthetic construct
  source 1..19: mol_type = other DNA
tacggcgaccaccgagatc

SEQ ID NO: 6 - DNA, 22 bp, synthetic construct
  source 1..22: mol_type = other DNA
aagcagtggtatcaacgcagag

SEQ ID NO: 7-8 - skipped (2 entries)

SEQ ID NO: 9 - DNA, 29 bp, synthetic construct
  source 1..29: mol_type = other DNA
aatgatacggcgaccaccgagatctacac

SEQ ID NO: 10 - DNA, 51 bp, synthetic construct
  source 1..51: mol_type = other DNA
caagcagaagacggcatacgagatcgtgatgtgactggagttcagacgtgt

SEQ ID NO: 11 - DNA, 51 bp, synthetic construct
  source 1..51: mol_type = other DNA
caagcagaagacggcatacgagatacatcggtgactggagttcagacgtgt

SEQ ID NO: 12 - DNA, 51 bp, synthetic construct
  source 1..51: mol_type = other DNA
caagcagaagacggcatacgagatgcctaagtgactggagttcagacgtgt

SEQ ID NO: 13 - DNA, 51 bp, synthetic construct
  source 1..51: mol_type = other DNA
caagcagaagacggcatacgagattggtcagtgactggagttcagacgtgt

SEQ ID NO: 14 - DNA, 51 bp, synthetic construct
  source 1..51: mol_type = other DNA
caagcagaagacggcatacgagatcactgtgtgactggagttcagacgtgt

SEQ ID NO: 15 - DNA, 51 bp, synthetic construct
  source 1..51: mol_type = other DNA
caagcagaagacggcatacgagatcagtgggtgactggagttcagacgtgt

SEQ ID NO: 16 - DNA, 51 bp, synthetic construct
  source 1..51: mol_type = other DNA
caagcagaagacggcatacgagatgttgtcgtgactggagttcagacgtgt

SEQ ID NO: 17 - DNA, 51 bp, synthetic construct
  source 1..51: mol_type = other DNA
caagcagaagacggcatacgagattgacaagtgactggagttcagacgtgt